European Patent Application EP 4 494 653 A1, published January 22, 2025. Title: PRLR ANTIGEN-BINDING PROTEIN, PREPARATION METHOD THEREFOR AND USE THEREOF. Applicant: Shenyang Sunshine Pharmaceutical Co., LTD. The sequence listing filed with the application follows.

SEQUENCE LISTING (21 sequences)

SEQ ID NO: 1 - protein, 210 aa, Artificial sequence
QLPPGKPEIFKCRSPNKETFTCWWRPGTDGGLPTNYSLTYHREGETLMHECPDYITGGPNSCHFGKQYTSMWRTYIMMVNATNQMGSSFSDELYVDVTYIVQPDPPLELAVEVKQPEDRKPYLWIKWSPPTLIDLKTGWFTLLYEIRLKPEKAAEWEIHFAGQQTEFKILSLHPGQKYLVQVRCKPDHGYWSAWSPATFIQIPSDFTMND

SEQ ID NO: 2 - protein, 120 aa, Artificial sequence
QVQLKESGPGLVAPSQSLSITCTVSGFSLTRNGVSWVRQPPGKGLEWLGIIWGDGSTNYHSALISRLSISKDNSKSQVFLKLNSLQTDDTATYYCAKEGLYYYGRYFDVWGAGTTVTVSS

SEQ ID NO: 3 - DNA, 360 bp, Artificial sequence
  source 1..360: mol_type = other DNA
caggtgcagctgaaggagtcaggacctggcctggtggcgccctcacagagcctgtccatcacatgcactgtctcagggttttcattaaccagaaatggtgtaagctgggttcgccagcctccaggaaagggtctggaatggctgggaataatatggggtgacgggagcacaaattatcattcagctctcatatccagactgagcatcagcaaggataactccaagagccaagttttcttaaaactgaacagtctgcaaactgatgacacagccacttactactgtgccaaagagggcctttattactacggacggtacttcgatgtctggggcgcagggaccacggtcaccgtctcctca

SEQ ID NO: 4 - protein, 107 aa, artificial sequence
DIVMTQSHKFMSTSVGDRVSITCKASQDVGSAVAWYQQKPGQSPKVLIYWASTRHTGVPDRFTGSGSGTDFTLTISNVQSEDLADYFCQQYSNYPLTFGGGTKLEIR

SEQ ID NO: 5 - DNA, 321 bp, Artificial sequence
  source 1..321: mol_type = other DNA
gacattgtgatgacccagtctcacaaattcatgtccacatcagtaggagacagggtcagcatcacctgcaaggccagtcaggatgtgggtagtgctgtagcctggtatcaacagaaaccagggcaatctcctaaagtactgatttactgggcatccacccggcacactggagtccctgatcgcttcacaggcagtggatctgggacagatttcactctcaccattagcaatgtgcagtctgaagacttggcagattatttctgtcagcaatatagcaactatcctctcacgttcggaggggggaccaagctggaaataaga

SEQ ID NO: 6 - protein, 330 aa, Artificial sequence [sequence omitted]

SEQ ID NO: 7 - protein, 107 aa, Artificial sequence [sequence omitted]

SEQ ID NO: 8 - protein, 450 aa, Artificial sequence
QVQLKESGPGLVAPSQSLSITCTVSGFSLTRNGVSWVRQPPGKGLEWLGIIWGDGSTNYHSALISRLSISKDNSKSQVFLKLNSLQTDDTATYYCAKEGLYYYGRYFDVWGAGTTVTVSSASTKGPSVFPLAPSSKSTSGGTAALGCLVKDYFPEPVTVSWNSGALTSGVHTFPAVLQSSGLYSLSSVVTVPSSSLGTQTYICNVNHKPSNTKVDKKVEPKSCDKTHTCPPCPAPELLGGPSVFLFPPKPKDTLMISRTPEVTCVVVDVSHEDPEVKFNWYVDGVEVHNAKTKPREEQYNSTYRVVSVLTVLHQDWLNGKEYKCKVSNKALPAPIEKTISKAKGQPREPQVYTLPPSRDELTKNQVSLTCLVKGFYPSDIAVEWESNGQPENNYKTTPPVLDSDGSFFLYSKLTVDKSRWQQGNVFSCSVMHEALHNHYTQKSLSLSPGK

SEQ ID NO: 9 - protein, 214 aa, Artificial sequence
DIVMTQSHKFMSTSVGDRVSITCKASQDVGSAVAWYQQKPGQSPKVLIYWASTRHTGVPDRFTGSGSGTDFTLTISNVQSEDLADYFCQQYSNYPLTFGGGTKLEIRRTVAAPSVFIFPPSDEQLKSGTASVVCLLNNFYPREAKVQWKVDNALQSGNSQESVTEQDSKDSTYSLSSTLTLSKADYEKHKVYACEVTHQGLSSPVTKSFNRGEC

SEQ ID NO: 10 - protein, 102 aa, Artificial sequence
PPGKPEIFKCRSPNKETFTCWWRPGTDGGLPTNYSLTYHREGETLMHECPDYITGGPNSCHFGKQYTSMWRTYIMMVNATNQMGSSFSDELYVDVTYIVQPD

SEQ ID NO: 11 - protein, 106 aa, Artificial sequence
PPLELAVEVKQPEDRKPYLWIKWSPPTLIDLKTGWFTLLYEIRLKPEKAAEWEIHFAGQQTEFKILSLHPGQKYLVQVRCKPDHGYWSAWSPATFIQIPSDFTMND

SEQ ID NO: 12 - protein, 12 aa, Artificial sequence
TVSGFSLTRNGV

SEQ ID NO: 13 - protein, 7 aa, Artificial sequence
IWGDGST

SEQ ID NO: 14 - protein, 14 aa, Artificial sequence
AKEGLYYYGRYFDV

SEQ ID NO: 15 - protein, 10 aa, Artificial sequence
KASQDVGSAV

SEQ ID NO: 16 - protein, 7 aa, Artificial sequence
WASTRHT

SEQ ID NO: 17 - protein, 9 aa, Artificial sequence
QQYSNYPLT

SEQ ID NO: 18 - protein, 120 aa, Artificial sequence
QVQLQESGPGLVKPSETLSLTCTVSGFSLTRNGVSWIRQPPGKGLEWVGVIWGDGSTNYNSAFMSRVTISVDTSKNQVSLKLSSVTAADTAVYYCAKEGLYYYGRYFDVWGQGTTVTVSS

SEQ ID NO: 19 - protein, 107 aa, Artificial sequence
DIQMTQSPSSLSASVGDRVTITCRASQDVGSALAWYQQKPGKVPKLLIYWASTRHTGVPSRFSGSGSGTDFTLTISSLQPEDVATYYCQQYSNYPLTFGGGTKLEIK

SEQ ID NO: 20 - protein, 450 aa, Artificial sequence
QVQLQESGPGLVKPSETLSLTCTVSGFSLTRNGVSWIRQPPGKGLEWVGVIWGDGSTNYNSAFMSRVTISVDTSKNQVSLKLSSVTAADTAVYYCAKEGLYYYGRYFDVWGQGTTVTVSSASTKGPSVFPLAPSSKSTSGGTAALGCLVKDYFPEPVTVSWNSGALTSGVHTFPAVLQSSGLYSLSSVVTVPSSSLGTQTYICNVNHKPSNTKVDKKVEPKSCDKTHTCPPCPAPELLGGPSVFLFPPKPKDTLMISRTPEVTCVVVDVSHEDPEVKFNWYVDGVEVHNAKTKPREEQYNSTYRVVSVLTVLHQDWLNGKEYKCKVSNKALPAPIEKTISKAKGQPREPQVYTLPPSRDELTKNQVSLTCLVKGFYPSDIAVEWESNGQPENNYKTTPPVLDSDGSFFLYSKLTVDKSRWQQGNVFSCSVMHEALHNHYTQKSLSLSPGK

SEQ ID NO: 21 - protein, 214 aa, Artificial sequence
DIQMTQSPSSLSASVGDRVTITCRASQDVGSALAWYQQKPGKVPKLLIYWASTRHTGVPSRFSGSGSGTDFTLTISSLQPEDVATYYCQQYSNYPLTFGGGTKLEIKRTVAAPSVFIFPPSDEQLKSGTASVVCLLNNFYPREAKVQWKVDNALQSGNSQESVTEQDSKDSTYSLSSTLTLSKADYEKHKVYACEVTHQGLSSPVTKSFNRGEC